European Patent Application EP 4 737 571 A1, published May 6, 2026. Title: 水痘带状疱疹病毒(VZV)疫苗. Applicant: 深圳深信生物科技有限公司. The sequence listing filed with the application follows.

SEQUENCE LISTING (35 sequences)

SEQ ID NO: 1 - protein, 623 aa, synthetic construct
MGTVNKPVVGVLMGFGIITGTLRITNPVRASVLRYDDFHIDEDKLDTNSVYEPYYHSDHAESSWVNRGESSRKAYDHNSPYIWPRNDYDGFLENAHEHHGVYNQGRGIDSGERLMQPTQMSAQEDLGDDTGIHVIPTLNGDDRHKIVNVDQRQYGDVFKGDLNPKPQGQRLIEVSVEENHPFTLRAPIQRIYGVRYTETWSFLPSLTCTGDAAPAIQHICLKHTTCFQDVVVDVDCAENTKEDQLAEISYRFQGKKEADQPWIVVNTSTLFDELELDPPEIEPGVLKVLRTEKQYLGVYIWNMRGSDGTSTYATFLVTWKGDEKTRNPTPAVTPQPRGAEFHMWNYHSHVFSVGDTFSLAMHLQYKIHEAPFDLLLEWLYVPIDPTCQPMRLYSTCLYHPNAPQCLSHMNSGCTFTSPHLAQRVASTVYQNCEHADNYTAYCLGISHMEPSFGLILHDGGTTLKFVDTPESLSGLYVFVVYFNGHVEAVAYTVVSTVDHFVNAIEERGFPPTAGQPPATTKPKEITPVNPGTSPLLRYAAWTGGLAAVVLLCLVIFLICTAKRMRVKAYRVDKSPYNQSMYYAGLPVDDFEDSESTDTEEEFGNAIGGSHGGSSYTVYIDKTR

SEQ ID NO: 2 - protein, 601 aa, synthetic construct
RITNPVRASVLRYDDFHIDEDKLDTNSVYEPYYHSDHAESSWVNRGESSRKAYDHNSPYIWPRNDYDGFLENAHEHHGVYNQGRGIDSGERLMQPTQMSAQEDLGDDTGIHVIPTLNGDDRHKIVNVDQRQYGDVFKGDLNPKPQGQRLIEVSVEENHPFTLRAPIQRIYGVRYTETWSFLPSLTCTGDAAPAIQHICLKHTTCFQDVVVDVDCAENTKEDQLAEISYRFQGKKEADQPWIVVNTSTLFDELELDPPEIEPGVLKVLRTEKQYLGVYIWNMRGSDGTSTYATFLVTWKGDEKTRNPTPAVTPQPRGAEFHMWNYHSHVFSVGDTFSLAMHLQYKIHEAPFDLLLEWLYVPIDPTCQPMRLYSTCLYHPNAPQCLSHMNSGCTFTSPHLAQRVASTVYQNCEHADNYTAYCLGISHMEPSFGLILHDGGTTLKFVDTPESLSGLYVFVVYFNGHVEAVAYTVVSTVDHFVNAIEERGFPPTAGQPPATTKPKEITPVNPGTSPLLRYAAWTGGLAAVVLLCLVIFLICTAKRMRVKAYRVDKSPYNQSMYYAGLPVDDFEDSESTDTEEEFGNAIGGSHGGSSYTVYIDKTR

SEQ ID NO: 3 - protein, 593 aa, synthetic construct
SVLRYDDFHIDEDKLDTNSVYEPYYHSDHAESSWVNRGESSRKAYDHNSPYIWPRNDYDGFLENAHEHHGVYNQGRGIDSGERLMQPTQMSAQEDLGDDTGIHVIPTLNGDDRHKIVNVDQRQYGDVFKGDLNPKPQGQRLIEVSVEENHPFTLRAPIQRIYGVRYTETWSFLPSLTCTGDAAPAIQHICLKHTTCFQDVVVDVDCAENTKEDQLAEISYRFQGKKEADQPWIVVNTSTLFDELELDPPEIEPGVLKVLRTEKQYLGVYIWNMRGSDGTSTYATFLVTWKGDEKTRNPTPAVTPQPRGAEFHMWNYHSHVFSVGDTFSLAMHLQYKIHEAPFDLLLEWLYVPIDPTCQPMRLYSTCLYHPNAPQCLSHMNSGCTFTSPHLAQRVASTVYQNCEHADNYTAYCLGISHMEPSFGLILHDGGTTLKFVDTPESLSGLYVFVVYFNGHVEAVAYTVVSTVDHFVNAIEERGFPPTAGQPPATTKPKEITPVNPGTSPLLRYAAWTGGLAAVVLLCLVIFLICTAKRMRVKAYRVDKSPYNQSMYYAGLPVDDFEDSESTDTEEEFGNAIGGSHGGSSYTVYIDKTR

SEQ ID NO: 4 - protein, 561 aa, synthetic construct
MGTVNKPVVGVLMGFGIITGTLRITNPVRASVLRYDDFHIDEDKLDTNSVYEPYYHSDHAESSWVNRGESSRKAYDHNSPYIWPRNDYDGFLENAHEHHGVYNQGRGIDSGERLMQPTQMSAQEDLGDDTGIHVIPTLNGDDRHKIVNVDQRQYGDVFKGDLNPKPQGQRLIEVSVEENHPFTLRAPIQRIYGVRYTETWSFLPSLTCTGDAAPAIQHICLKHTTCFQDVVVDVDCAENTKEDQLAEISYRFQGKKEADQPWIVVNTSTLFDELELDPPEIEPGVLKVLRTEKQYLGVYIWNMRGSDGTSTYATFLVTWKGDEKTRNPTPAVTPQPRGAEFHMWNYHSHVFSVGDTFSLAMHLQYKIHEAPFDLLLEWLYVPIDPTCQPMRLYSTCLYHPNAPQCLSHMNSGCTFTSPHLAQRVASTVYQNCEHADNYTAYCLGISHMEPSFGLILHDGGTTLKFVDTPESLSGLYVFVVYFNGHVEAVAYTVVSTVDHFVNAIEERGFPPTAGQPPATTKPKEITPVNPGTSPLLRYAAWTGGLAAVVLLCLVIFLICTA

SEQ ID NO: 5 - protein, 573 aa, synthetic construct
MGTVNKPVVGVLMGFGIITGTLRITNPVRASVLRYDDFHIDEDKLDTNSVYEPYYHSDHAESSWVNRGESSRKAYDHNSPYIWPRNDYDGFLENAHEHHGVYNQGRGIDSGERLMQPTQMSAQEDLGDDTGIHVIPTLNGDDRHKIVNVDQRQYGDVFKGDLNPKPQGQRLIEVSVEENHPFTLRAPIQRIYGVRYTETWSFLPSLTCTGDAAPAIQHICLKHTTCFQDVVVDVDCAENTKEDQLAEISYRFQGKKEADQPWIVVNTSTLFDELELDPPEIEPGVLKVLRTEKQYLGVYIWNMRGSDGTSTYATFLVTWKGDEKTRNPTPAVTPQPRGAEFHMWNYHSHVFSVGDTFSLAMHLQYKIHEAPFDLLLEWLYVPIDPTCQPMRLYSTCLYHPNAPQCLSHMNSGCTFTSPHLAQRVASTVYQNCEHADNYTAYCLGISHMEPSFGLILHDGGTTLKFVDTPESLSGLYVFVVYFNGHVEAVAYTVVSTVDHFVNAIEERGFPPTAGQPPATTKPKEITPVNPGTSPLLRYAAWTGGLAAVVLLCLVIFLICTAKRMRVKAARVDK

SEQ ID NO: 6 - protein, 543 aa, synthetic construct
MGTVNKPVVGVLMGFGIITGTLRITNPVRASVLRYDDFHIDEDKLDTNSVYEPYYHSDHAESSWVNRGESSRKAYDHNSPYIWPRNDYDGFLENAHEHHGVYNQGRGIDSGERLMQPTQMSAQEDLGDDTGIHVIPTLNGDDRHKIVNVDQRQYGDVFKGDLNPKPQGQRLIEVSVEENHPFTLRAPIQRIYGVRYTETWSFLPSLTCTGDAAPAIQHICLKHTTCFQDVVVDVDCAENTKEDQLAEISYRFQGKKEADQPWIVVNTSTLFDELELDPPEIEPGVLKVLRTEKQYLGVYIWNMRGSDGTSTYATFLVTWKGDEKTRNPTPAVTPQPRGAEFHMWNYHSHVFSVGDTFSLAMHLQYKIHEAPFDLLLEWLYVPIDPTCQPMRLYSTCLYHPNAPQCLSHMNSGCTFTSPHLAQRVASTVYQNCEHADNYTAYCLGISHMEPSFGLILHDGGTTLKFVDTPESLSGLYVFVVYFNGHVEAVAYTVVSTVDHFVNAIEERGFPPTAGQPPATTKPKEITPVNPGTSPLLRYAAWTG

SEQ ID NO: 7 - protein, 543 aa, synthetic construct
SVLRYDDFHIDEDKLDTNSVYEPYYHSDHAESSWVNRGESSRKAYDHNSPYIWPRNDYDGFLENAHEHHGVYNQGRGIDSGERLMQPTQMSAQEDLGDDTGIHVIPTLNGDDRHKIVNVDQRQYGDVFKGDLNPKPQGQRLIEVSVEENHPFTLRAPIQRIYGVRYTETWSFLPSLTCTGDAAPAIQHICLKHTTCFQDVVVDVDCAENTKEDQLAEISYRFQGKKEADQPWIVVNTSTLFDELELDPPEIEPGVLKVLRTEKQYLGVYIWNMRGSDGTSTYATFLVTWKGDEKTRNPTPAVTPQPRGAEFHMWNYHSHVFSVGDTFSLAMHLQYKIHEAPFDLLLEWLYVPIDPTCQPMRLYSTCLYHPNAPQCLSHMNSGCTFTSPHLAQRVASTVYQNCEHADNYTAYCLGISHMEPSFGLILHDGGTTLKFVDTPESLSGLYVFVVYFNGHVEAVAYTVVSTVDHFVNAIEERGFPPTAGQPPATTKPKEITPVNPGTSPLLRYAAWTGGLAAVVLLCLVIFLICTAKRMRVKAARVDK

SEQ ID NO: 8 - protein, 513 aa, synthetic construct
SVLRYDDFHIDEDKLDTNSVYEPYYHSDHAESSWVNRGESSRKAYDHNSPYIWPRNDYDGFLENAHEHHGVYNQGRGIDSGERLMQPTQMSAQEDLGDDTGIHVIPTLNGDDRHKIVNVDQRQYGDVFKGDLNPKPQGQRLIEVSVEENHPFTLRAPIQRIYGVRYTETWSFLPSLTCTGDAAPAIQHICLKHTTCFQDVVVDVDCAENTKEDQLAEISYRFQGKKEADQPWIVVNTSTLFDELELDPPEIEPGVLKVLRTEKQYLGVYIWNMRGSDGTSTYATFLVTWKGDEKTRNPTPAVTPQPRGAEFHMWNYHSHVFSVGDTFSLAMHLQYKIHEAPFDLLLEWLYVPIDPTCQPMRLYSTCLYHPNAPQCLSHMNSGCTFTSPHLAQRVASTVYQNCEHADNYTAYCLGISHMEPSFGLILHDGGTTLKFVDTPESLSGLYVFVVYFNGHVEAVAYTVVSTVDHFVNAIEERGFPPTAGQPPATTKPKEITPVNPGTSPLLRYAAWTG

SEQ ID NO: 9 - protein, 20 aa, synthetic construct
METDTLLLWVLLLWVPGSTG

SEQ ID NO: 10 - protein, 174 aa, synthetic construct
MESQVRQQFSKDIEKLLNEQVNKEMNSSNLYMSMSSWCYTHSLDGAGLFLFDHAAEEYEHAKKLIIFLNENNVPVQLTSISAPEHKFEGLTQIFQKAYEHEQHISESINNIVDHAIKSKDHATFNFLQWYVAEQHEEEVLFKDILDKIELIGNENHGLYLADQYVKGIAKSRKS

SEQ ID NO: 11 - DNA, 1872 bp, synthetic construct
  source 1..1872: mol_type = other DNA
atgggcacagtgaacaagcctgttgtgggcgtgctgatgggcttcggcatcatcacaggcaccctgagaatcaccaatcctgtgcgggccagcgtgctgagatacgacgatttccacatcgacgaggacaagctggacaccaacagcgtgtacgagccctactaccacagcgatcacgccgagtctagctgggtcaacagaggcgaaagcagcagaaaggcctacgaccacaacagcccctacatctggcccagaaacgactacgacggcttcctggaaaatgcccacgaacaccacggcgtgtacaatcaaggcagaggcatcgatagcggcgagagactgatgcagcctacacagatgagcgcccaagaggatctgggcgacgatacaggcatccacgtgatccctacactgaacggcgacgaccggcacaagatcgtgaatgtggatcagagacagtacggcgacgtgttcaagggcgatctgaaccctaagcctcagggccagcgcctgatcgaagtgtccgtggaagaaaatcaccccttcacactgagagcccctatccagagaatctacggcgtgcgctataccgagacatggtcctttctgcctagcctgacatgtactggcgacgccgctcctgccatccagcacatttgtctgaagcacaccacctgtttccaggacgtggtggtggatgtggactgcgccgagaacaccaaagaggatcagctggccgagatcagctaccggttccagggaaagaaagaggccgaccagccttggatcgtggtcaacaccagcacactgttcgacgagctggaactggaccctcctgagattgagcctggggtgctgaaggtgctgagaaccgagaagcagtacctgggagtgtacatctggaacatgagaggctccgacggcaccagcacctacgccacatttctggttacctggaagggcgacgaaaagaccagaaatcccacaccagccgtgacacctcaacctagaggcgccgagtttcacatgtggaattaccacagccacgtgttcagcgtgggcgatacctttagcctggccatgcatctgcagtacaagatccacgaggcccctttcgacctgctgctggaatggctgtacgtgcccatcgatcctacctgccagcctatgagactgtacagcacctgtctgtatcaccccaacgctcctcagtgcctgagccacatgaatagcggctgcaccttcacaagccctcacctggctcagagagtggccagcacagtctaccagaattgcgagcacgccgacaattacaccgcctactgtctgggcatcagccacatggaacctagcttcggcctgatcctgcacgatggcggcaccacactgaagttcgtggatacacctgagagcctgagcggcctgtatgtgtttgtggtgtacttcaacggccacgtggaagccgtggcctacactgtggtgtccaccgtggatcacttcgtgaacgccatcgaggaacggggatttccaccaactgctggacagcctcctgccaccaccaagcctaaagaaatcacacccgtgaatcccggcacctctccactgcttagatatgccgcttggacaggcggactggctgctgtggttctgctgtgcctggtcatcttcctgatctgcaccgccaagcggatgagagtgaaggcctacagagtggacaagagcccttacaaccagagcatgtactacgccggcctgcctgtggacgatttcgaggatagcgagagcaccgacaccgaggaagagtttggcaacgccattggaggctctcacggcggcagcagctacaccgtgtacatcgacaagacccggtga

SEQ ID NO: 12 - DNA, 1806 bp, synthetic construct
  source 1..1806: mol_type = other DNA
agaatcaccaatcctgtgcgggccagcgtgctgagatacgacgatttccacatcgacgaggacaagctggacaccaacagcgtgtacgagccctactaccacagcgatcacgccgagtctagctgggtcaacagaggcgaaagcagcagaaaggcctacgaccacaacagcccctacatctggcccagaaacgactacgacggcttcctggaaaatgcccacgaacaccacggcgtgtacaatcaaggcagaggcatcgatagcggcgagagactgatgcagcctacacagatgagcgcccaagaggatctgggcgacgatacaggcatccacgtgatccctacactgaacggcgacgaccggcacaagatcgtgaatgtggatcagagacagtacggcgacgtgttcaagggcgatctgaaccctaagcctcagggccagcgcctgatcgaagtgtccgtggaagaaaatcaccccttcacactgagagcccctatccagagaatctacggcgtgcgctataccgagacatggtcctttctgcctagcctgacatgtactggcgacgccgctcctgccatccagcacatttgtctgaagcacaccacctgtttccaggacgtggtggtggatgtggactgcgccgagaacaccaaagaggatcagctggccgagatcagctaccggttccagggaaagaaagaggccgaccagccttggatcgtggtcaacaccagcacactgttcgacgagctggaactggaccctcctgagattgagcctggggtgctgaaggtgctgagaaccgagaagcagtacctgggagtgtacatctggaacatgagaggctccgacggcaccagcacctacgccacatttctggttacctggaagggcgacgaaaagaccagaaatcccacaccagccgtgacacctcaacctagaggcgccgagtttcacatgtggaattaccacagccacgtgttcagcgtgggcgatacctttagcctggccatgcatctgcagtacaagatccacgaggcccctttcgacctgctgctggaatggctgtacgtgcccatcgatcctacctgccagcctatgagactgtacagcacctgtctgtatcaccccaacgctcctcagtgcctgagccacatgaatagcggctgcaccttcacaagccctcacctggctcagagagtggccagcacagtctaccagaattgcgagcacgccgacaattacaccgcctactgtctgggcatcagccacatggaacctagcttcggcctgatcctgcacgatggcggcaccacactgaagttcgtggatacacctgagagcctgagcggcctgtatgtgtttgtggtgtacttcaacggccacgtggaagccgtggcctacactgtggtgtccaccgtggatcacttcgtgaacgccatcgaggaacggggatttccaccaactgctggacagcctcctgccaccaccaagcctaaagaaatcacacccgtgaatcccggcacctctccactgcttagatatgccgcttggacaggcggactggctgctgtggttctgctgtgcctggtcatcttcctgatctgcaccgccaagcggatgagagtgaaggcctacagagtggacaagagcccttacaaccagagcatgtactacgccggcctgcctgtggacgatttcgaggatagcgagagcaccgacaccgaggaagagtttggcaacgccattggaggctctcacggcggcagcagctacaccgtgtacatcgacaagacccggtga

SEQ ID NO: 13 - DNA, 1782 bp, synthetic construct
  source 1..1782: mol_type = other DNA
agcgtgctgagatacgacgatttccacatcgacgaggacaagctggacaccaacagcgtgtacgagccctactaccacagcgatcacgccgagtctagctgggtcaacagaggcgaaagcagcagaaaggcctacgaccacaacagcccctacatctggcccagaaacgactacgacggcttcctggaaaatgcccacgaacaccacggcgtgtacaatcaaggcagaggcatcgatagcggcgagagactgatgcagcctacacagatgagcgcccaagaggatctgggcgacgatacaggcatccacgtgatccctacactgaacggcgacgaccggcacaagatcgtgaatgtggatcagagacagtacggcgacgtgttcaagggcgatctgaaccctaagcctcagggccagcgcctgatcgaagtgtccgtggaagaaaatcaccccttcacactgagagcccctatccagagaatctacggcgtgcgctataccgagacatggtcctttctgcctagcctgacatgtactggcgacgccgctcctgccatccagcacatttgtctgaagcacaccacctgtttccaggacgtggtggtggatgtggactgcgccgagaacaccaaagaggatcagctggccgagatcagctaccggttccagggaaagaaagaggccgaccagccttggatcgtggtcaacaccagcacactgttcgacgagctggaactggaccctcctgagattgagcctggggtgctgaaggtgctgagaaccgagaagcagtacctgggagtgtacatctggaacatgagaggctccgacggcaccagcacctacgccacatttctggttacctggaagggcgacgaaaagaccagaaatcccacaccagccgtgacacctcaacctagaggcgccgagtttcacatgtggaattaccacagccacgtgttcagcgtgggcgatacctttagcctggccatgcatctgcagtacaagatccacgaggcccctttcgacctgctgctggaatggctgtacgtgcccatcgatcctacctgccagcctatgagactgtacagcacctgtctgtatcaccccaacgctcctcagtgcctgagccacatgaatagcggctgcaccttcacaagccctcacctggctcagagagtggccagcacagtctaccagaattgcgagcacgccgacaattacaccgcctactgtctgggcatcagccacatggaacctagcttcggcctgatcctgcacgatggcggcaccacactgaagttcgtggatacacctgagagcctgagcggcctgtatgtgtttgtggtgtacttcaacggccacgtggaagccgtggcctacactgtggtgtccaccgtggatcacttcgtgaacgccatcgaggaacggggatttccaccaactgctggacagcctcctgccaccaccaagcctaaagaaatcacacccgtgaatcccggcacctctccactgcttagatatgccgcttggacaggcggactggctgctgtggttctgctgtgcctggtcatcttcctgatctgcaccgccaagcggatgagagtgaaggcctacagagtggacaagagcccttacaaccagagcatgtactacgccggcctgcctgtggacgatttcgaggatagcgagagcaccgacaccgaggaagagtttggcaacgccattggaggctctcacggcggcagcagctacaccgtgtacatcgacaagacccggtga

SEQ ID NO: 14 - DNA, 1686 bp, synthetic construct
  source 1..1686: mol_type = other DNA
atgggcacagtgaacaagcctgttgtgggcgtgctgatgggcttcggcatcatcacaggcaccctgagaatcaccaatcctgtgcgggccagcgtgctgagatacgacgatttccacatcgacgaggacaagctggacaccaacagcgtgtacgagccctactaccacagcgatcacgccgagtctagctgggtcaacagaggcgaaagcagcagaaaggcctacgaccacaacagcccctacatctggcccagaaacgactacgacggcttcctggaaaatgcccacgaacaccacggcgtgtacaatcaaggcagaggcatcgatagcggcgagagactgatgcagcctacacagatgagcgcccaagaggatctgggcgacgatacaggcatccacgtgatccctacactgaacggcgacgaccggcacaagatcgtgaatgtggatcagagacagtacggcgacgtgttcaagggcgatctgaaccctaagcctcagggccagcgcctgatcgaagtgtccgtggaagaaaatcaccccttcacactgagagcccctatccagagaatctacggcgtgcgctataccgagacatggtcctttctgcctagcctgacatgtactggcgacgccgctcctgccatccagcacatttgtctgaagcacaccacctgtttccaggacgtggtggtggatgtggactgcgccgagaacaccaaagaggatcagctggccgagatcagctaccggttccagggaaagaaagaggccgaccagccttggatcgtggtcaacaccagcacactgttcgacgagctggaactggaccctcctgagattgagcctggggtgctgaaggtgctgagaaccgagaagcagtacctgggagtgtacatctggaacatgagaggctccgacggcaccagcacctacgccacatttctggttacctggaagggcgacgaaaagaccagaaatcccacaccagccgtgacacctcaacctagaggcgccgagtttcacatgtggaattaccacagccacgtgttcagcgtgggcgatacctttagcctggccatgcatctgcagtacaagatccacgaggcccctttcgacctgctgctggaatggctgtacgtgcccatcgatcctacctgccagcctatgagactgtacagcacctgtctgtatcaccccaacgctcctcagtgcctgagccacatgaatagcggctgcaccttcacaagccctcacctggctcagagagtggccagcacagtctaccagaattgcgagcacgccgacaattacaccgcctactgtctgggcatcagccacatggaacctagcttcggcctgatcctgcacgatggcggcaccacactgaagttcgtggatacacctgagagcctgagcggcctgtatgtgtttgtggtgtacttcaacggccacgtggaagccgtggcctacactgtggtgtccaccgtggatcacttcgtgaacgccatcgaggaacggggatttccaccaactgctggacagcctcctgccaccaccaagcctaaagaaatcacacccgtgaatcccggcacctctccactgcttagatatgccgcttggacaggcggactggctgctgtggttctgctgtgcctggtcatcttcctgatctgcaccgcctga

SEQ ID NO: 15 - DNA, 1722 bp, synthetic construct
  source 1..1722: mol_type = other DNA
atgggcacagtgaacaagcctgttgtgggcgtgctgatgggcttcggcatcatcacaggcaccctgagaatcaccaatcctgtgcgggccagcgtgctgagatacgacgatttccacatcgacgaggacaagctggacaccaacagcgtgtacgagccctactaccacagcgatcacgccgagtctagctgggtcaacagaggcgaaagcagcagaaaggcctacgaccacaacagcccctacatctggcccagaaacgactacgacggcttcctggaaaatgcccacgaacaccacggcgtgtacaatcaaggcagaggcatcgatagcggcgagagactgatgcagcctacacagatgagcgcccaagaggatctgggcgacgatacaggcatccacgtgatccctacactgaacggcgacgaccggcacaagatcgtgaatgtggatcagagacagtacggcgacgtgttcaagggcgatctgaaccctaagcctcagggccagcgcctgatcgaagtgtccgtggaagaaaatcaccccttcacactgagagcccctatccagagaatctacggcgtgcgctataccgagacatggtcctttctgcctagcctgacatgtactggcgacgccgctcctgccatccagcacatttgtctgaagcacaccacctgtttccaggacgtggtggtggatgtggactgcgccgagaacaccaaagaggatcagctggccgagatcagctaccggttccagggaaagaaagaggccgaccagccttggatcgtggtcaacaccagcacactgttcgacgagctggaactggaccctcctgagattgagcctggggtgctgaaggtgctgagaaccgagaagcagtacctgggagtgtacatctggaacatgagaggctccgacggcaccagcacctacgccacatttctggttacctggaagggcgacgaaaagaccagaaatcccacaccagccgtgacacctcaacctagaggcgccgagtttcacatgtggaattaccacagccacgtgttcagcgtgggcgatacctttagcctggccatgcatctgcagtacaagatccacgaggcccctttcgacctgctgctggaatggctgtacgtgcccatcgatcctacctgccagcctatgagactgtacagcacctgtctgtatcaccccaacgctcctcagtgcctgagccacatgaatagcggctgcaccttcacaagccctcacctggctcagagagtggccagcacagtctaccagaattgcgagcacgccgacaattacaccgcctactgtctgggcatcagccacatggaacctagcttcggcctgatcctgcacgatggcggcaccacactgaagttcgtggatacacctgagagcctgagcggcctgtatgtgtttgtggtgtacttcaacggccacgtggaagccgtggcctacactgtggtgtccaccgtggatcacttcgtgaacgccatcgaggaacggggatttccaccaactgctggacagcctcctgccaccaccaagcctaaagaaatcacacccgtgaatcccggcacctctccactgcttagatatgccgcttggacaggcggactggctgctgtggttctgctgtgcctggtcatcttcctgatctgcaccgccaagcggatgagagtgaaggccgcaagagtggacaagtga

SEQ ID NO: 16 - DNA, 1632 bp, synthetic construct
  source 1..1632: mol_type = other DNA
atgggcacagtgaacaagcctgttgtgggcgtgctgatgggcttcggcatcatcacaggcaccctgagaatcaccaatcctgtgcgggccagcgtgctgagatacgacgatttccacatcgacgaggacaagctggacaccaacagcgtgtacgagccctactaccacagcgatcacgccgagtctagctgggtcaacagaggcgaaagcagcagaaaggcctacgaccacaacagcccctacatctggcccagaaacgactacgacggcttcctggaaaatgcccacgaacaccacggcgtgtacaatcaaggcagaggcatcgatagcggcgagagactgatgcagcctacacagatgagcgcccaagaggatctgggcgacgatacaggcatccacgtgatccctacactgaacggcgacgaccggcacaagatcgtgaatgtggatcagagacagtacggcgacgtgttcaagggcgatctgaaccctaagcctcagggccagcgcctgatcgaagtgtccgtggaagaaaatcaccccttcacactgagagcccctatccagagaatctacggcgtgcgctataccgagacatggtcctttctgcctagcctgacatgtactggcgacgccgctcctgccatccagcacatttgtctgaagcacaccacctgtttccaggacgtggtggtggatgtggactgcgccgagaacaccaaagaggatcagctggccgagatcagctaccggttccagggaaagaaagaggccgaccagccttggatcgtggtcaacaccagcacactgttcgacgagctggaactggaccctcctgagattgagcctggggtgctgaaggtgctgagaaccgagaagcagtacctgggagtgtacatctggaacatgagaggctccgacggcaccagcacctacgccacatttctggttacctggaagggcgacgaaaagaccagaaatcccacaccagccgtgacacctcaacctagaggcgccgagtttcacatgtggaattaccacagccacgtgttcagcgtgggcgatacctttagcctggccatgcatctgcagtacaagatccacgaggcccctttcgacctgctgctggaatggctgtacgtgcccatcgatcctacctgccagcctatgagactgtacagcacctgtctgtatcaccccaacgctcctcagtgcctgagccacatgaatagcggctgcaccttcacaagccctcacctggctcagagagtggccagcacagtctaccagaattgcgagcacgccgacaattacaccgcctactgtctgggcatcagccacatggaacctagcttcggcctgatcctgcacgatggcggcaccacactgaagttcgtggatacacctgagagcctgagcggcctgtatgtgtttgtggtgtacttcaacggccacgtggaagccgtggcctacactgtggtgtccaccgtggatcacttcgtgaacgccatcgaggaacggggatttccaccaactgctggacagcctcctgccaccaccaagcctaaagaaatcacacccgtgaatcccggcacctctccactgcttagatatgccgcttggacaggctga

SEQ ID NO: 17 - DNA, 1632 bp, synthetic construct
  source 1..1632: mol_type = other DNA
agcgtgctgagatacgacgatttccacatcgacgaggacaagctggacaccaacagcgtgtacgagccctactaccacagcgatcacgccgagtctagctgggtcaacagaggcgaaagcagcagaaaggcctacgaccacaacagcccctacatctggcccagaaacgactacgacggcttcctggaaaatgcccacgaacaccacggcgtgtacaatcaaggcagaggcatcgatagcggcgagagactgatgcagcctacacagatgagcgcccaagaggatctgggcgacgatacaggcatccacgtgatccctacactgaacggcgacgaccggcacaagatcgtgaatgtggatcagagacagtacggcgacgtgttcaagggcgatctgaaccctaagcctcagggccagcgcctgatcgaagtgtccgtggaagaaaatcaccccttcacactgagagcccctatccagagaatctacggcgtgcgctataccgagacatggtcctttctgcctagcctgacatgtactggcgacgccgctcctgccatccagcacatttgtctgaagcacaccacctgtttccaggacgtggtggtggatgtggactgcgccgagaacaccaaagaggatcagctggccgagatcagctaccggttccagggaaagaaagaggccgaccagccttggatcgtggtcaacaccagcacactgttcgacgagctggaactggaccctcctgagattgagcctggggtgctgaaggtgctgagaaccgagaagcagtacctgggagtgtacatctggaacatgagaggctccgacggcaccagcacctacgccacatttctggttacctggaagggcgacgaaaagaccagaaatcccacaccagccgtgacacctcaacctagaggcgccgagtttcacatgtggaattaccacagccacgtgttcagcgtgggcgatacctttagcctggccatgcatctgcagtacaagatccacgaggcccctttcgacctgctgctggaatggctgtacgtgcccatcgatcctacctgccagcctatgagactgtacagcacctgtctgtatcaccccaacgctcctcagtgcctgagccacatgaatagcggctgcaccttcacaagccctcacctggctcagagagtggccagcacagtctaccagaattgcgagcacgccgacaattacaccgcctactgtctgggcatcagccacatggaacctagcttcggcctgatcctgcacgatggcggcaccacactgaagttcgtggatacacctgagagcctgagcggcctgtatgtgtttgtggtgtacttcaacggccacgtggaagccgtggcctacactgtggtgtccaccgtggatcacttcgtgaacgccatcgaggaacggggatttccaccaactgctggacagcctcctgccaccaccaagcctaaagaaatcacacccgtgaatcccggcacctctccactgcttagatatgccgcttggacaggcggactggctgctgtggttctgctgtgcctggtcatcttcctgatctgcaccgccaagcggatgagagtgaaggccgcaagagtggacaagtga

SEQ ID NO: 18 - DNA, 1542 bp, synthetic construct
  source 1..1542: mol_type = other DNA
agcgtgctgagatacgacgatttccacatcgacgaggacaagctggacaccaacagcgtgtacgagccctactaccacagcgatcacgccgagtctagctgggtcaacagaggcgaaagcagcagaaaggcctacgaccacaacagcccctacatctggcccagaaacgactacgacggcttcctggaaaatgcccacgaacaccacggcgtgtacaatcaaggcagaggcatcgatagcggcgagagactgatgcagcctacacagatgagcgcccaagaggatctgggcgacgatacaggcatccacgtgatccctacactgaacggcgacgaccggcacaagatcgtgaatgtggatcagagacagtacggcgacgtgttcaagggcgatctgaaccctaagcctcagggccagcgcctgatcgaagtgtccgtggaagaaaatcaccccttcacactgagagcccctatccagagaatctacggcgtgcgctataccgagacatggtcctttctgcctagcctgacatgtactggcgacgccgctcctgccatccagcacatttgtctgaagcacaccacctgtttccaggacgtggtggtggatgtggactgcgccgagaacaccaaagaggatcagctggccgagatcagctaccggttccagggaaagaaagaggccgaccagccttggatcgtggtcaacaccagcacactgttcgacgagctggaactggaccctcctgagattgagcctggggtgctgaaggtgctgagaaccgagaagcagtacctgggagtgtacatctggaacatgagaggctccgacggcaccagcacctacgccacatttctggttacctggaagggcgacgaaaagaccagaaatcccacaccagccgtgacacctcaacctagaggcgccgagtttcacatgtggaattaccacagccacgtgttcagcgtgggcgatacctttagcctggccatgcatctgcagtacaagatccacgaggcccctttcgacctgctgctggaatggctgtacgtgcccatcgatcctacctgccagcctatgagactgtacagcacctgtctgtatcaccccaacgctcctcagtgcctgagccacatgaatagcggctgcaccttcacaagccctcacctggctcagagagtggccagcacagtctaccagaattgcgagcacgccgacaattacaccgcctactgtctgggcatcagccacatggaacctagcttcggcctgatcctgcacgatggcggcaccacactgaagttcgtggatacacctgagagcctgagcggcctgtatgtgtttgtggtgtacttcaacggccacgtggaagccgtggcctacactgtggtgtccaccgtggatcacttcgtgaacgccatcgaggaacggggatttccaccaactgctggacagcctcctgccaccaccaagcctaaagaaatcacacccgtgaatcccggcacctctccactgcttagatatgccgcttggacaggctga

SEQ ID NO: 19 - DNA, 1932 bp, synthetic construct
  source 1..1932: mol_type = other DNA
atggagacagacacactcctgctatgggtgctgctgctctgggttccaggttccacaggtatgggcacagtgaacaagcctgttgtgggcgtgctgatgggcttcggcatcatcacaggcaccctgagaatcaccaatcctgtgcgggccagcgtgctgagatacgacgatttccacatcgacgaggacaagctggacaccaacagcgtgtacgagccctactaccacagcgatcacgccgagtctagctgggtcaacagaggcgaaagcagcagaaaggcctacgaccacaacagcccctacatctggcccagaaacgactacgacggcttcctggaaaatgcccacgaacaccacggcgtgtacaatcaaggcagaggcatcgatagcggcgagagactgatgcagcctacacagatgagcgcccaagaggatctgggcgacgatacaggcatccacgtgatccctacactgaacggcgacgaccggcacaagatcgtgaatgtggatcagagacagtacggcgacgtgttcaagggcgatctgaaccctaagcctcagggccagcgcctgatcgaagtgtccgtggaagaaaatcaccccttcacactgagagcccctatccagagaatctacggcgtgcgctataccgagacatggtcctttctgcctagcctgacatgtactggcgacgccgctcctgccatccagcacatttgtctgaagcacaccacctgtttccaggacgtggtggtggatgtggactgcgccgagaacaccaaagaggatcagctggccgagatcagctaccggttccagggaaagaaagaggccgaccagccttggatcgtggtcaacaccagcacactgttcgacgagctggaactggaccctcctgagattgagcctggggtgctgaaggtgctgagaaccgagaagcagtacctgggagtgtacatctggaacatgagaggctccgacggcaccagcacctacgccacatttctggttacctggaagggcgacgaaaagaccagaaatcccacaccagccgtgacacctcaacctagaggcgccgagtttcacatgtggaattaccacagccacgtgttcagcgtgggcgatacctttagcctggccatgcatctgcagtacaagatccacgaggcccctttcgacctgctgctggaatggctgtacgtgcccatcgatcctacctgccagcctatgagactgtacagcacctgtctgtatcaccccaacgctcctcagtgcctgagccacatgaatagcggctgcaccttcacaagccctcacctggctcagagagtggccagcacagtctaccagaattgcgagcacgccgacaattacaccgcctactgtctgggcatcagccacatggaacctagcttcggcctgatcctgcacgatggcggcaccacactgaagttcgtggatacacctgagagcctgagcggcctgtatgtgtttgtggtgtacttcaacggccacgtggaagccgtggcctacactgtggtgtccaccgtggatcacttcgtgaacgccatcgaggaacggggatttccaccaactgctggacagcctcctgccaccaccaagcctaaagaaatcacacccgtgaatcccggcacctctccactgcttagatatgccgcttggacaggcggactggctgctgtggttctgctgtgcctggtcatcttcctgatctgcaccgccaagcggatgagagtgaaggcctacagagtggacaagagcccttacaaccagagcatgtactacgccggcctgcctgtggacgatttcgaggatagcgagagcaccgacaccgaggaagagtttggcaacgccattggaggctctcacggcggcagcagctacaccgtgtacatcgacaagacccggtga

SEQ ID NO: 20 - DNA, 1866 bp, synthetic construct
  source 1..1866: mol_type = other DNA
atggagacagacacactcctgctatgggtgctgctgctctgggttccaggttccacaggtagaatcaccaatcctgtgcgggccagcgtgctgagatacgacgatttccacatcgacgaggacaagctggacaccaacagcgtgtacgagccctactaccacagcgatcacgccgagtctagctgggtcaacagaggcgaaagcagcagaaaggcctacgaccacaacagcccctacatctggcccagaaacgactacgacggcttcctggaaaatgcccacgaacaccacggcgtgtacaatcaaggcagaggcatcgatagcggcgagagactgatgcagcctacacagatgagcgcccaagaggatctgggcgacgatacaggcatccacgtgatccctacactgaacggcgacgaccggcacaagatcgtgaatgtggatcagagacagtacggcgacgtgttcaagggcgatctgaaccctaagcctcagggccagcgcctgatcgaagtgtccgtggaagaaaatcaccccttcacactgagagcccctatccagagaatctacggcgtgcgctataccgagacatggtcctttctgcctagcctgacatgtactggcgacgccgctcctgccatccagcacatttgtctgaagcacaccacctgtttccaggacgtggtggtggatgtggactgcgccgagaacaccaaagaggatcagctggccgagatcagctaccggttccagggaaagaaagaggccgaccagccttggatcgtggtcaacaccagcacactgttcgacgagctggaactggaccctcctgagattgagcctggggtgctgaaggtgctgagaaccgagaagcagtacctgggagtgtacatctggaacatgagaggctccgacggcaccagcacctacgccacatttctggttacctggaagggcgacgaaaagaccagaaatcccacaccagccgtgacacctcaacctagaggcgccgagtttcacatgtggaattaccacagccacgtgttcagcgtgggcgatacctttagcctggccatgcatctgcagtacaagatccacgaggcccctttcgacctgctgctggaatggctgtacgtgcccatcgatcctacctgccagcctatgagactgtacagcacctgtctgtatcaccccaacgctcctcagtgcctgagccacatgaatagcggctgcaccttcacaagccctcacctggctcagagagtggccagcacagtctaccagaattgcgagcacgccgacaattacaccgcctactgtctgggcatcagccacatggaacctagcttcggcctgatcctgcacgatggcggcaccacactgaagttcgtggatacacctgagagcctgagcggcctgtatgtgtttgtggtgtacttcaacggccacgtggaagccgtggcctacactgtggtgtccaccgtggatcacttcgtgaacgccatcgaggaacggggatttccaccaactgctggacagcctcctgccaccaccaagcctaaagaaatcacacccgtgaatcccggcacctctccactgcttagatatgccgcttggacaggcggactggctgctgtggttctgctgtgcctggtcatcttcctgatctgcaccgccaagcggatgagagtgaaggcctacagagtggacaagagcccttacaaccagagcatgtactacgccggcctgcctgtggacgatttcgaggatagcgagagcaccgacaccgaggaagagtttggcaacgccattggaggctctcacggcggcagcagctacaccgtgtacatcgacaagacccggtga

SEQ ID NO: 21 - DNA, 1842 bp, synthetic construct
  source 1..1842: mol_type = other DNA
atggagacagacacactcctgctatgggtgctgctgctctgggttccaggttccacaggtagcgtgctgagatacgacgatttccacatcgacgaggacaagctggacaccaacagcgtgtacgagccctactaccacagcgatcacgccgagtctagctgggtcaacagaggcgaaagcagcagaaaggcctacgaccacaacagcccctacatctggcccagaaacgactacgacggcttcctggaaaatgcccacgaacaccacggcgtgtacaatcaaggcagaggcatcgatagcggcgagagactgatgcagcctacacagatgagcgcccaagaggatctgggcgacgatacaggcatccacgtgatccctacactgaacggcgacgaccggcacaagatcgtgaatgtggatcagagacagtacggcgacgtgttcaagggcgatctgaaccctaagcctcagggccagcgcctgatcgaagtgtccgtggaagaaaatcaccccttcacactgagagcccctatccagagaatctacggcgtgcgctataccgagacatggtcctttctgcctagcctgacatgtactggcgacgccgctcctgccatccagcacatttgtctgaagcacaccacctgtttccaggacgtggtggtggatgtggactgcgccgagaacaccaaagaggatcagctggccgagatcagctaccggttccagggaaagaaagaggccgaccagccttggatcgtggtcaacaccagcacactgttcgacgagctggaactggaccctcctgagattgagcctggggtgctgaaggtgctgagaaccgagaagcagtacctgggagtgtacatctggaacatgagaggctccgacggcaccagcacctacgccacatttctggttacctggaagggcgacgaaaagaccagaaatcccacaccagccgtgacacctcaacctagaggcgccgagtttcacatgtggaattaccacagccacgtgttcagcgtgggcgatacctttagcctggccatgcatctgcagtacaagatccacgaggcccctttcgacctgctgctggaatggctgtacgtgcccatcgatcctacctgccagcctatgagactgtacagcacctgtctgtatcaccccaacgctcctcagtgcctgagccacatgaatagcggctgcaccttcacaagccctcacctggctcagagagtggccagcacagtctaccagaattgcgagcacgccgacaattacaccgcctactgtctgggcatcagccacatggaacctagcttcggcctgatcctgcacgatggcggcaccacactgaagttcgtggatacacctgagagcctgagcggcctgtatgtgtttgtggtgtacttcaacggccacgtggaagccgtggcctacactgtggtgtccaccgtggatcacttcgtgaacgccatcgaggaacggggatttccaccaactgctggacagcctcctgccaccaccaagcctaaagaaatcacacccgtgaatcccggcacctctccactgcttagatatgccgcttggacaggcggactggctgctgtggttctgctgtgcctggtcatcttcctgatctgcaccgccaagcggatgagagtgaaggcctacagagtggacaagagcccttacaaccagagcatgtactacgccggcctgcctgtggacgatttcgaggatagcgagagcaccgacaccgaggaagagtttggcaacgccattggaggctctcacggcggcagcagctacaccgtgtacatcgacaagacccggtga

SEQ ID NO: 22 - DNA, 2169 bp, synthetic construct
  source 1..2169: mol_type = other DNA
atgggcacagtgaacaagcctgttgtgggcgtgctgatgggcttcggcatcatcacaggcaccctgagaatcaccaatcctgtgcgggccagcgtgctgagatacgacgatttccacatcgacgaggacaagctggacaccaacagcgtgtacgagccctactaccacagcgatcacgccgagtctagctgggtcaacagaggcgaaagcagcagaaaggcctacgaccacaacagcccctacatctggcccagaaacgactacgacggcttcctggaaaatgcccacgaacaccacggcgtgtacaatcaaggcagaggcatcgatagcggcgagagactgatgcagcctacacagatgagcgcccaagaggatctgggcgacgatacaggcatccacgtgatccctacactgaacggcgacgaccggcacaagatcgtgaatgtggatcagagacagtacggcgacgtgttcaagggcgatctgaaccctaagcctcagggccagcgcctgatcgaagtgtccgtggaagaaaatcaccccttcacactgagagcccctatccagagaatctacggcgtgcgctataccgagacatggtcctttctgcctagcctgacatgtactggcgacgccgctcctgccatccagcacatttgtctgaagcacaccacctgtttccaggacgtggtggtggatgtggactgcgccgagaacaccaaagaggatcagctggccgagatcagctaccggttccagggaaagaaagaggccgaccagccttggatcgtggtcaacaccagcacactgttcgacgagctggaactggaccctcctgagattgagcctggggtgctgaaggtgctgagaaccgagaagcagtacctgggagtgtacatctggaacatgagaggctccgacggcaccagcacctacgccacatttctggttacctggaagggcgacgaaaagaccagaaatcccacaccagccgtgacacctcaacctagaggcgccgagtttcacatgtggaattaccacagccacgtgttcagcgtgggcgatacctttagcctggccatgcatctgcagtacaagatccacgaggcccctttcgacctgctgctggaatggctgtacgtgcccatcgatcctacctgccagcctatgagactgtacagcacctgtctgtatcaccccaacgctcctcagtgcctgagccacatgaatagcggctgcaccttcacaagccctcacctggctcagagagtggccagcacagtctaccagaattgcgagcacgccgacaattacaccgcctactgtctgggcatcagccacatggaacctagcttcggcctgatcctgcacgatggcggcaccacactgaagttcgtggatacacctgagagcctgagcggcctgtatgtgtttgtggtgtacttcaacggccacgtggaagccgtggcctacactgtggtgtccaccgtggatcacttcgtgaacgccatcgaggaacggggatttccaccaactgctggacagcctcctgccaccaccaagcctaaagaaatcacacccgtgaatcccggcacctctccactgcttagatatgccgcttggacaggcagcgccatcggcatggaatctcaagtgcggcagcagttcagcaaggacatcgagaagctgctgaacgagcaagtgaacaaagagatgaacagcagcaacctgtacatgagcatgagcagctggtgctacacccacagtctggatggcgccggactgttcctgtttgatcacgccgccgaggaatacgagcacgccaagaagctgatcatcttcctgaacgagaacaacgtgcccgtgcagctgacatctatcagcgcccctgagcacaagttcgagggcctgacacagatcttccagaaggcctacgaacacgagcagcacatcagcgagagcatcaacaacatcgtggaccacgccatcaagagcaaggatcacgccaccttcaactttctgcagtggtacgtggccgaacagcacgaggaagaggtgctgtttaaggacatcctggacaagatcgagctgatcggcaacgagaaccacggcctgtacctggccgatcagtatgtgaagggaatcgccaagagccggaagtcctgatga

SEQ ID NO: 23 - DNA, 1692 bp, synthetic construct
  source 1..1692: mol_type = other DNA
atggagacagacacactcctgctatgggtgctgctgctctgggttccaggttccacaggtagcgtgctgagatacgacgatttccacatcgacgaggacaagctggacaccaacagcgtgtacgagccctactaccacagcgatcacgccgagtctagctgggtcaacagaggcgaaagcagcagaaaggcctacgaccacaacagcccctacatctggcccagaaacgactacgacggcttcctggaaaatgcccacgaacaccacggcgtgtacaatcaaggcagaggcatcgatagcggcgagagactgatgcagcctacacagatgagcgcccaagaggatctgggcgacgatacaggcatccacgtgatccctacactgaacggcgacgaccggcacaagatcgtgaatgtggatcagagacagtacggcgacgtgttcaagggcgatctgaaccctaagcctcagggccagcgcctgatcgaagtgtccgtggaagaaaatcaccccttcacactgagagcccctatccagagaatctacggcgtgcgctataccgagacatggtcctttctgcctagcctgacatgtactggcgacgccgctcctgccatccagcacatttgtctgaagcacaccacctgtttccaggacgtggtggtggatgtggactgcgccgagaacaccaaagaggatcagctggccgagatcagctaccggttccagggaaagaaagaggccgaccagccttggatcgtggtcaacaccagcacactgttcgacgagctggaactggaccctcctgagattgagcctggggtgctgaaggtgctgagaaccgagaagcagtacctgggagtgtacatctggaacatgagaggctccgacggcaccagcacctacgccacatttctggttacctggaagggcgacgaaaagaccagaaatcccacaccagccgtgacacctcaacctagaggcgccgagtttcacatgtggaattaccacagccacgtgttcagcgtgggcgatacctttagcctggccatgcatctgcagtacaagatccacgaggcccctttcgacctgctgctggaatggctgtacgtgcccatcgatcctacctgccagcctatgagactgtacagcacctgtctgtatcaccccaacgctcctcagtgcctgagccacatgaatagcggctgcaccttcacaagccctcacctggctcagagagtggccagcacagtctaccagaattgcgagcacgccgacaattacaccgcctactgtctgggcatcagccacatggaacctagcttcggcctgatcctgcacgatggcggcaccacactgaagttcgtggatacacctgagagcctgagcggcctgtatgtgtttgtggtgtacttcaacggccacgtggaagccgtggcctacactgtggtgtccaccgtggatcacttcgtgaacgccatcgaggaacggggatttccaccaactgctggacagcctcctgccaccaccaagcctaaagaaatcacacccgtgaatcccggcacctctccactgcttagatatgccgcttggacaggcggactggctgctgtggttctgctgtgcctggtcatcttcctgatctgcaccgccaagcggatgagagtgaaggccgcaagagtggacaagtga

SEQ ID NO: 24 - DNA, 2139 bp, synthetic construct
  source 1..2139: mol_type = other DNA
atggagacagacacactcctgctatgggtgctgctgctctgggttccaggttccacaggtagcgtgctgagatacgacgatttccacatcgacgaggacaagctggacaccaacagcgtgtacgagccctactaccacagcgatcacgccgagtctagctgggtcaacagaggcgaaagcagcagaaaggcctacgaccacaacagcccctacatctggcccagaaacgactacgacggcttcctggaaaatgcccacgaacaccacggcgtgtacaatcaaggcagaggcatcgatagcggcgagagactgatgcagcctacacagatgagcgcccaagaggatctgggcgacgatacaggcatccacgtgatccctacactgaacggcgacgaccggcacaagatcgtgaatgtggatcagagacagtacggcgacgtgttcaagggcgatctgaaccctaagcctcagggccagcgcctgatcgaagtgtccgtggaagaaaatcaccccttcacactgagagcccctatccagagaatctacggcgtgcgctataccgagacatggtcctttctgcctagcctgacatgtactggcgacgccgctcctgccatccagcacatttgtctgaagcacaccacctgtttccaggacgtggtggtggatgtggactgcgccgagaacaccaaagaggatcagctggccgagatcagctaccggttccagggaaagaaagaggccgaccagccttggatcgtggtcaacaccagcacactgttcgacgagctggaactggaccctcctgagattgagcctggggtgctgaaggtgctgagaaccgagaagcagtacctgggagtgtacatctggaacatgagaggctccgacggcaccagcacctacgccacatttctggttacctggaagggcgacgaaaagaccagaaatcccacaccagccgtgacacctcaacctagaggcgccgagtttcacatgtggaattaccacagccacgtgttcagcgtgggcgatacctttagcctggccatgcatctgcagtacaagatccacgaggcccctttcgacctgctgctggaatggctgtacgtgcccatcgatcctacctgccagcctatgagactgtacagcacctgtctgtatcaccccaacgctcctcagtgcctgagccacatgaatagcggctgcaccttcacaagccctcacctggctcagagagtggccagcacagtctaccagaattgcgagcacgccgacaattacaccgcctactgtctgggcatcagccacatggaacctagcttcggcctgatcctgcacgatggcggcaccacactgaagttcgtggatacacctgagagcctgagcggcctgtatgtgtttgtggtgtacttcaacggccacgtggaagccgtggcctacactgtggtgtccaccgtggatcacttcgtgaacgccatcgaggaacggggatttccaccaactgctggacagcctcctgccaccaccaagcctaaagaaatcacacccgtgaatcccggcacctctccactgcttagatatgccgcttggacaggcagcgccatcggcatggaatctcaagtgcggcagcagttcagcaaggacatcgagaagctgctgaacgagcaagtgaacaaagagatgaacagcagcaacctgtacatgagcatgagcagctggtgctacacccacagtctggatggcgccggactgttcctgtttgatcacgccgccgaggaatacgagcacgccaagaagctgatcatcttcctgaacgagaacaacgtgcccgtgcagctgacatctatcagcgcccctgagcacaagttcgagggcctgacacagatcttccagaaggcctacgaacacgagcagcacatcagcgagagcatcaacaacatcgtggaccacgccatcaagagcaaggatcacgccaccttcaactttctgcagtggtacgtggccgaacagcacgaggaagaggtgctgtttaaggacatcctggacaagatcgagctgatcggcaacgagaaccacggcctgtacctggccgatcagtatgtgaagggaatcgccaagagccggaagtcctgatga

SEQ ID NO: 25 - DNA, 170 bp, synthetic construct
  source 1..170: mol_type = other DNA
taatacgactcactataggacagatcgcctggagacgccatccacgctgttttgacctccatagaagacaccgggaccgatccagcctccgcggccgggaacggtgcattggaacgcggattccccgtgccaagagtgacgtaagtaccgcagtcaccgtccttgacacg

SEQ ID NO: 26 - DNA, 74 bp, synthetic construct
  source 1..74: mol_type = other DNA
tcttcacccagtctgtctcttagaatttatttcccactgacacaaacaagccattttgtctgcttgtataaccc

SEQ ID NO: 27 - DNA, 106 bp, synthetic construct
  source 1..106: mol_type = other DNA
aaaaaaaaaaaagaaaaaaaaaaaaaaaaaagaaagaaaaaaaaaaaaaaaaaaaaaaaaaaaaaaaaaaaaaaaaaaaaaaaaaaaaaaaaaaaaaaaaaaaaaa

SEQ ID NO: 28 - protein, 643 aa, synthetic construct
METDTLLLWVLLLWVPGSTGMGTVNKPVVGVLMGFGIITGTLRITNPVRASVLRYDDFHIDEDKLDTNSVYEPYYHSDHAESSWVNRGESSRKAYDHNSPYIWPRNDYDGFLENAHEHHGVYNQGRGIDSGERLMQPTQMSAQEDLGDDTGIHVIPTLNGDDRHKIVNVDQRQYGDVFKGDLNPKPQGQRLIEVSVEENHPFTLRAPIQRIYGVRYTETWSFLPSLTCTGDAAPAIQHICLKHTTCFQDVVVDVDCAENTKEDQLAEISYRFQGKKEADQPWIVVNTSTLFDELELDPPEIEPGVLKVLRTEKQYLGVYIWNMRGSDGTSTYATFLVTWKGDEKTRNPTPAVTPQPRGAEFHMWNYHSHVFSVGDTFSLAMHLQYKIHEAPFDLLLEWLYVPIDPTCQPMRLYSTCLYHPNAPQCLSHMNSGCTFTSPHLAQRVASTVYQNCEHADNYTAYCLGISHMEPSFGLILHDGGTTLKFVDTPESLSGLYVFVVYFNGHVEAVAYTVVSTVDHFVNAIEERGFPPTAGQPPATTKPKEITPVNPGTSPLLRYAAWTGGLAAVVLLCLVIFLICTAKRMRVKAYRVDKSPYNQSMYYAGLPVDDFEDSESTDTEEEFGNAIGGSHGGSSYTVYIDKTR

SEQ ID NO: 29 - protein, 621 aa, synthetic construct
METDTLLLWVLLLWVPGSTGRITNPVRASVLRYDDFHIDEDKLDTNSVYEPYYHSDHAESSWVNRGESSRKAYDHNSPYIWPRNDYDGFLENAHEHHGVYNQGRGIDSGERLMQPTQMSAQEDLGDDTGIHVIPTLNGDDRHKIVNVDQRQYGDVFKGDLNPKPQGQRLIEVSVEENHPFTLRAPIQRIYGVRYTETWSFLPSLTCTGDAAPAIQHICLKHTTCFQDVVVDVDCAENTKEDQLAEISYRFQGKKEADQPWIVVNTSTLFDELELDPPEIEPGVLKVLRTEKQYLGVYIWNMRGSDGTSTYATFLVTWKGDEKTRNPTPAVTPQPRGAEFHMWNYHSHVFSVGDTFSLAMHLQYKIHEAPFDLLLEWLYVPIDPTCQPMRLYSTCLYHPNAPQCLSHMNSGCTFTSPHLAQRVASTVYQNCEHADNYTAYCLGISHMEPSFGLILHDGGTTLKFVDTPESLSGLYVFVVYFNGHVEAVAYTVVSTVDHFVNAIEERGFPPTAGQPPATTKPKEITPVNPGTSPLLRYAAWTGGLAAVVLLCLVIFLICTAKRMRVKAYRVDKSPYNQSMYYAGLPVDDFEDSESTDTEEEFGNAIGGSHGGSSYTVYIDKTR

SEQ ID NO: 30 - protein, 613 aa, synthetic construct
METDTLLLWVLLLWVPGSTGSVLRYDDFHIDEDKLDTNSVYEPYYHSDHAESSWVNRGESSRKAYDHNSPYIWPRNDYDGFLENAHEHHGVYNQGRGIDSGERLMQPTQMSAQEDLGDDTGIHVIPTLNGDDRHKIVNVDQRQYGDVFKGDLNPKPQGQRLIEVSVEENHPFTLRAPIQRIYGVRYTETWSFLPSLTCTGDAAPAIQHICLKHTTCFQDVVVDVDCAENTKEDQLAEISYRFQGKKEADQPWIVVNTSTLFDELELDPPEIEPGVLKVLRTEKQYLGVYIWNMRGSDGTSTYATFLVTWKGDEKTRNPTPAVTPQPRGAEFHMWNYHSHVFSVGDTFSLAMHLQYKIHEAPFDLLLEWLYVPIDPTCQPMRLYSTCLYHPNAPQCLSHMNSGCTFTSPHLAQRVASTVYQNCEHADNYTAYCLGISHMEPSFGLILHDGGTTLKFVDTPESLSGLYVFVVYFNGHVEAVAYTVVSTVDHFVNAIEERGFPPTAGQPPATTKPKEITPVNPGTSPLLRYAAWTGGLAAVVLLCLVIFLICTAKRMRVKAYRVDKSPYNQSMYYAGLPVDDFEDSESTDTEEEFGNAIGGSHGGSSYTVYIDKTR

SEQ ID NO: 31 - protein, 721 aa, synthetic construct
MGTVNKPVVGVLMGFGIITGTLRITNPVRASVLRYDDFHIDEDKLDTNSVYEPYYHSDHAESSWVNRGESSRKAYDHNSPYIWPRNDYDGFLENAHEHHGVYNQGRGIDSGERLMQPTQMSAQEDLGDDTGIHVIPTLNGDDRHKIVNVDQRQYGDVFKGDLNPKPQGQRLIEVSVEENHPFTLRAPIQRIYGVRYTETWSFLPSLTCTGDAAPAIQHICLKHTTCFQDVVVDVDCAENTKEDQLAEISYRFQGKKEADQPWIVVNTSTLFDELELDPPEIEPGVLKVLRTEKQYLGVYIWNMRGSDGTSTYATFLVTWKGDEKTRNPTPAVTPQPRGAEFHMWNYHSHVFSVGDTFSLAMHLQYKIHEAPFDLLLEWLYVPIDPTCQPMRLYSTCLYHPNAPQCLSHMNSGCTFTSPHLAQRVASTVYQNCEHADNYTAYCLGISHMEPSFGLILHDGGTTLKFVDTPESLSGLYVFVVYFNGHVEAVAYTVVSTVDHFVNAIEERGFPPTAGQPPATTKPKEITPVNPGTSPLLRYAAWTGSAIGMESQVRQQFSKDIEKLLNEQVNKEMNSSNLYMSMSSWCYTHSLDGAGLFLFDHAAEEYEHAKKLIIFLNENNVPVQLTSISAPEHKFEGLTQIFQKAYEHEQHISESINNIVDHAIKSKDHATFNFLQWYVAEQHEEEVLFKDILDKIELIGNENHGLYLADQYVKGIAKSRKS

SEQ ID NO: 32 - protein, 563 aa, synthetic construct
METDTLLLWVLLLWVPGSTGSVLRYDDFHIDEDKLDTNSVYEPYYHSDHAESSWVNRGESSRKAYDHNSPYIWPRNDYDGFLENAHEHHGVYNQGRGIDSGERLMQPTQMSAQEDLGDDTGIHVIPTLNGDDRHKIVNVDQRQYGDVFKGDLNPKPQGQRLIEVSVEENHPFTLRAPIQRIYGVRYTETWSFLPSLTCTGDAAPAIQHICLKHTTCFQDVVVDVDCAENTKEDQLAEISYRFQGKKEADQPWIVVNTSTLFDELELDPPEIEPGVLKVLRTEKQYLGVYIWNMRGSDGTSTYATFLVTWKGDEKTRNPTPAVTPQPRGAEFHMWNYHSHVFSVGDTFSLAMHLQYKIHEAPFDLLLEWLYVPIDPTCQPMRLYSTCLYHPNAPQCLSHMNSGCTFTSPHLAQRVASTVYQNCEHADNYTAYCLGISHMEPSFGLILHDGGTTLKFVDTPESLSGLYVFVVYFNGHVEAVAYTVVSTVDHFVNAIEERGFPPTAGQPPATTKPKEITPVNPGTSPLLRYAAWTGGLAAVVLLCLVIFLICTAKRMRVKAARVDK

SEQ ID NO: 33 - protein, 711 aa, synthetic construct
METDTLLLWVLLLWVPGSTGSVLRYDDFHIDEDKLDTNSVYEPYYHSDHAESSWVNRGESSRKAYDHNSPYIWPRNDYDGFLENAHEHHGVYNQGRGIDSGERLMQPTQMSAQEDLGDDTGIHVIPTLNGDDRHKIVNVDQRQYGDVFKGDLNPKPQGQRLIEVSVEENHPFTLRAPIQRIYGVRYTETWSFLPSLTCTGDAAPAIQHICLKHTTCFQDVVVDVDCAENTKEDQLAEISYRFQGKKEADQPWIVVNTSTLFDELELDPPEIEPGVLKVLRTEKQYLGVYIWNMRGSDGTSTYATFLVTWKGDEKTRNPTPAVTPQPRGAEFHMWNYHSHVFSVGDTFSLAMHLQYKIHEAPFDLLLEWLYVPIDPTCQPMRLYSTCLYHPNAPQCLSHMNSGCTFTSPHLAQRVASTVYQNCEHADNYTAYCLGISHMEPSFGLILHDGGTTLKFVDTPESLSGLYVFVVYFNGHVEAVAYTVVSTVDHFVNAIEERGFPPTAGQPPATTKPKEITPVNPGTSPLLRYAAWTGSAIGMESQVRQQFSKDIEKLLNEQVNKEMNSSNLYMSMSSWCYTHSLDGAGLFLFDHAAEEYEHAKKLIIFLNENNVPVQLTSISAPEHKFEGLTQIFQKAYEHEQHISESINNIVDHAIKSKDHATFNFLQWYVAEQHEEEVLFKDILDKIELIGNENHGLYLADQYVKGIAKSRKS

SEQ ID NO: 34 - DNA, 60 bp, synthetic construct
  source 1..60: mol_type = other DNA
atggagacagacacactcctgctatgggtgctgctgctctgggttccaggttccacaggt

SEQ ID NO: 35 - DNA, 528 bp, synthetic construct
  source 1..528: mol_type = other DNA
atggaatctcaagtgcggcagcagttcagcaaggacatcgagaagctgctgaacgagcaagtgaacaaagagatgaacagcagcaacctgtacatgagcatgagcagctggtgctacacccacagtctggatggcgccggactgttcctgtttgatcacgccgccgaggaatacgagcacgccaagaagctgatcatcttcctgaacgagaacaacgtgcccgtgcagctgacatctatcagcgcccctgagcacaagttcgagggcctgacacagatcttccagaaggcctacgaacacgagcagcacatcagcgagagcatcaacaacatcgtggaccacgccatcaagagcaaggatcacgccaccttcaactttctgcagtggtacgtggccgaacagcacgaggaagaggtgctgtttaaggacatcctggacaagatcgagctgatcggcaacgagaaccacggcctgtacctggccgatcagtatgtgaagggaatcgccaagagccggaagtcctgatga